European Patent Application EP 4 249 097 A2, published September 27, 2023. Title: FC BINDING PROTEINS WITH CYSTEINE IN THE C-TERMINAL HELICAL REGION. Applicant: Repligen Corporation. The sequence listing filed with the application follows.

SEQUENCE LISTING (95 sequences)

SEQ ID NO: 1 - protein, 58 aa, synthetic construct
  REGION 1..58: note = consensus sequence 1
  SITE 1: note = variant - may be replaced by A, N, Q, V, or deleted
  SITE 2: note = variant - may be replaced by D or Q, or deleted
  SITE 3: note = variant - may be replaced by N, or deleted
  SITE 4: note = variant - may be replaced by Q or N, or deleted
  SITE 5: note = variant - may be replaced by F, or deleted
  SITE 6: note = variant - may be replaced by N, or deleted
  SITE 7: note = variant - may be replaced by E
  SITE 8: note = variant - may be replaced by A or E
  SITE 11: note = variant - may be replaced by S, N, I ,or E
  SITE 15: note = variant - may be replaced by Q
  SITE 16: note = variant - may be replaced by V
  SITE 18: note = variant - may be replaced by N
  SITE 19: note = variant - may be replaced by M
  SITE 23: note = variant - may be replaced by N
  SITE 24: note = variant - may be replaced by A
  SITE 25: note = variant - may be replaced by E
  SITE 29: note = variant - may be replaced by G
  SITE 35: note = variant - may be replaced by K or I
  SITE 40: note = variant - may be replaced by Q or T
  SITE 42: note = variant - may be replaced by A, K, or T
  SITE 43: note = variant - may be replaced by S, N, or C
  SITE 44: note = variant - may be replaced by L or V
  SITE 46: note = variant - may be replaced by C or A
  SITE 47: note = variant - may be replaced by C
  SITE 49: note = variant - may be replaced by Q
  SITE 50: note = variant - may be replaced by C
  SITE 51: note = variant - may be replaced by C
  SITE 53: note = variant - may be replaced by E or C
  SITE 54: note = variant - may be replaced by S, or deleted
  SITE 57: note = variant - may be deleted
  SITE 58: note = variant - may be replaced by K, or deleted
IAAKHDKDQQAAFYEILHLPNLTEDQRNAFIQSLRDDPSVSLEILGEAKKLNDAQAPP

SEQ ID NO: 2 - protein, 58 aa, synthetic construct; identical to SEQ ID NO: 1
  REGION 1..58: note = consensus sequence 2
  SITE 1: note = variant - may be deleted
  SITE 2: note = variant - may be replaced by D, or deleted
  SITE 3: note = variant - may be replaced by N or deleted
  SITE 4: note = variant - may be replaced by Q, or deleted
  SITE 5: note = variant - may be replaced by F, or deleted
  SITE 6: note = variant - may be deleted
  SITE 7: note = variant - may be replaced by E
  SITE 8: note = variant - may be replaced by A or E
  SITE 11: note = variant - may be replaced by S, I, or E
  SITE 25: note = variant - may be replaced by E
  SITE 35: note = variant - may be replaced by I
  SITE 40: note = variant - may be replaced by Q or T
  SITE 43: note = variant - may be replaced by S, or C
  SITE 44: note = variant - may be replaced by L or V
  SITE 46: note = variant - may be replaced by C or A
  SITE 47: note = variant - may be replaced by C
  SITE 49: note = variant - may be replaced by Q
  SITE 50: note = variant - may be replaced by C
  SITE 51: note = variant - may be replaced byC
  SITE 53: note = variant - may be replaced by E or C
  SITE 54: note = variant - may be replaced by S
  SITE 57: note = variant - may be deleted
  SITE 58: note = variant - may be replaced by K, or deleted

SEQ ID NO: 3 - protein, 58 aa, synthetic construct; identical to SEQ ID NO: 1
  REGION 1..58: note = cs14

SEQ ID NO: 4 - protein, 58 aa, synthetic construct
  REGION 1..58: note = cs27
IAAKFDEAQQAAFYEILHLPNLTEEQRNAFIQSLRDDPSVSLEVLGEAQKLNDSQAPK

SEQ ID NO: 5 - protein, 58 aa, synthetic construct
  REGION 1..58: note = cs20
IDSKFDEAQQAAFYEILHLPSLTEDQRNAFIQSLRDDPSTSLSLLGEAKKLNDAQAPP

SEQ ID NO: 6 - protein, 58 aa, synthetic construct
  REGION 1..58: note = cs42
IDAKHDEDQQAAFYEILHLPNLTEEQRNAFIQSLRDDPSQSLEILGEAKKLNESQAPK

SEQ ID NO: 7 - protein, 58 aa, synthetic construct
  REGION 1..58: note = cs26
IAAQHDKDQQAAFYEILHLPNLTEEQRNAFIQSLRDDPSVSLEILAEAKKLNDAQAPK

SEQ ID NO: 8 - protein, 58 aa, synthetic construct
  REGION 1..58: note = cs24
IAAQHDKEQQAAFYEILHLPNLTEDQRNAFIQSLRDDPSVSLEILGEAKKLNDAQAPK

SEQ ID NO: 9 - protein, 58 aa, synthetic construct
  REGION 1..58: note = cs17
IDSKFDEAQQAAFYEILHLPNLTEDQRNAFIQSLRDDPSVSLSLLGEAKKLNDAQAPP

SEQ ID NO: 10 - protein, 58 aa, synthetic construct
  REGION 1..58: note = cs25
IAAKHDKDQQAAFYEILHLPNLTEDQRNAFIQSLRDDPSVSLEILAEAKKLNDAQAPK

SEQ ID NO: 11 - protein, 58 aa, synthetic construct
  REGION 1..58: note = cs47h3
IAAKHDKDQQAAFYEILHLPNLTEDQRNAFIQSLRDDPSVSLEVLGEAQKLNDSQAPK

SEQ ID NO: 12 - protein, 58 aa, synthetic construct
  REGION 1..58: note = cs47h4
IAAKHDKDQQAAFYEILHLPNLTEEQRNAFIQSLRDDPSVSLEVLGEAQKLNDSQAPK

SEQ ID NO: 13 - protein, 58 aa, synthetic construct
  REGION 1..58: note = cs74h1
IAAKFDEAQQAAFYEILHLPNLTEDQRNAFIQSLRDDPSVSLEILGEAKKLNDAQAPP

SEQ ID NO: 14 - protein, 58 aa, synthetic construct
  REGION 1..58: note = cs74h2
IAAKFDEAQQAAFYEILHLPNLTEEQRNAFIQSLRDDPSVSLEILGEAKKLNDAQAPP

SEQ ID NO: 15 - protein, 58 aa, synthetic construct
  REGION 1..58: note = cs41
IAAKHDEDQQAAFYEILHLPNLTEEQRNAFIQSLRDDPSVSLEILGEAKKLNDSQAPK

SEQ ID NO: 16 - protein, 58 aa, synthetic construct
  REGION 1..58: note = cs43
IAAKHDKDQQAAFYEILHLPNLTEEQRNAFIQSLRDDPSVSLEILGEAKKLNDSQAPK

SEQ ID NO: 17 - protein, 58 aa, synthetic construct
  REGION 1..58: note = cs14 43C
IAAKHDKDQQAAFYEILHLPNLTEDQRNAFIQSLRDDPSVSLCILGEAKKLNDAQAPP

SEQ ID NO: 18 - protein, 58 aa, synthetic construct
  REGION 1..58: note = cs14 46C
IAAKHDKDQQAAFYEILHLPNLTEDQRNAFIQSLRDDPSVSLEILCEAKKLNDAQAPP

SEQ ID NO: 19 - protein, 58 aa, synthetic construct
  REGION 1..58: note = cs14 47C
IAAKHDKDQQAAFYEILHLPNLTEDQRNAFIQSLRDDPSVSLEILGCAKKLNDAQAPP

SEQ ID NO: 20 - protein, 58 aa, synthetic construct
  REGION 1..58: note = cs14 11S 46C
IAAKHDKDQQSAFYEILHLPNLTEDQRNAFIQSLRDDPSVSLEILCEAKKLNDAQAPP

SEQ ID NO: 21 - protein, 58 aa, synthetic construct
  REGION 1..58: note = cs27 43C
IAAKFDEAQQAAFYEILHLPNLTEEQRNAFIQSLRDDPSVSLCVLGEAQKLNDSQAPK

SEQ ID NO: 22 - protein, 58 aa, synthetic construct
  REGION 1..58: note = cs27 46C
IAAKFDEAQQAAFYEILHLPNLTEEQRNAFIQSLRDDPSVSLEVLCEAQKLNDSQAPK

SEQ ID NO: 23 - protein, 58 aa, synthetic construct
  REGION 1..58: note = cs27 47C
IAAKFDEAQQAAFYEILHLPNLTEEQRNAFIQSLRDDPSVSLEVLGCAQKLNDSQAPK

SEQ ID NO: 24 - protein, 58 aa, synthetic construct
  REGION 1..58: note = cs27 11S 46C
IAAKFDEAQQSAFYEILHLPNLTEEQRNAFIQSLRDDPSVSLEVLCEAQKLNDSQAPK

SEQ ID NO: 25 - protein, 116 aa, synthetic construct
  REGION 1..116: note = cs27 46C dimer
IAAKFDEAQQAAFYEILHLPNLTEEQRNAFIQSLRDDPSVSLEVLCEAQKLNDSQAPKIAAKFDEAQQAAFYEILHLPNLTEEQRNAFIQSLRDDPSVSLEVLCEAQKLNDSQAPK

SEQ ID NO: 26 - protein, 58 aa, synthetic construct
  REGION 1..58: note = cs26 43C
IAAQHDKDQQAAFYEILHLPNLTEEQRNAFIQSLRDDPSVSLCILAEAKKLNDAQAPK

SEQ ID NO: 27 - protein, 58 aa, synthetic construct
  REGION 1..58: note = cs26 46C
IAAQHDKDQQAAFYEILHLPNLTEEQRNAFIQSLRDDPSVSLEILCEAKKLNDAQAPK

SEQ ID NO: 28 - protein, 58 aa, synthetic construct
  REGION 1..58: note = cs26 47C
IAAQHDKDQQAAFYEILHLPNLTEEQRNAFIQSLRDDPSVSLEILACAKKLNDAQAPK

SEQ ID NO: 29 - protein, 58 aa, synthetic construct
  REGION 1..58: note = cs26 11S 46C
IAAQHDKDQQSAFYEILHLPNLTEEQRNAFIQSLRDDPSVSLEILCEAKKLNDAQAPK

SEQ ID NO: 30 - protein, 58 aa, synthetic construct
  REGION 1..58: note = cs26 9H 46C
IAAQHDKDHQAAFYEILHLPNLTEEQRNAFIQSLRDDPSVSLEILCEAKKLNDAQAPK

SEQ ID NO: 31 - protein, 58 aa, synthetic construct
  REGION 1..58: note = cs26 36H 46C
IAAQHDKDQQAAFYEILHLPNLTEEQRNAFIQSLRHDPSVSLEILCEAKKLNDAQAPK

SEQ ID NO: 32 - protein, 116 aa, synthetic construct
  REGION 1..116: note = cs26 46C dimer
IAAQHDKDQQAAFYEILHLPNLTEEQRNAFIQSLRDDPSVSLEILCEAKKLNDAQAPKIAAQHDKDQQAAFYEILHLPNLTEEQRNAFIQSLRDDPSVSLEILCEAKKLNDAQAPK

SEQ ID NO: 33 - protein, 55 aa, synthetic construct
  REGION 1..55: note = cs26 delN 46C
AHDKDQQAAFYEILHLPNLTEEQRNAFIQSLRDDPSVSLEILCEAKKLNDAQAPK

SEQ ID NO: 34 - protein, 53 aa, synthetic construct
  REGION 1..53: note = cs26 delNC 46C
QHDKDQQAAFYEILHLPNLTEEQRNAFIQSLRDDPSVSLEILCEAKKLNDAQA

SEQ ID NO: 35 - protein, 174 aa, synthetic construct
  REGION 1..174: note = cs26 46C trimer
IAAQHDKDQQAAFYEILHLPNLTEEQRNAFIQSLRDDPSVSLEILCEAKKLNDAQAPKIAAQHDKDQQAAFYEILHLPNLTEEQRNAFIQSLRDDPSVSLEILCEAKKLNDAQAPKIAAQHDKDQQAAFYEILHLPNLTEEQRNAFIQSLRDDPSVSLEILCEAKKLNDAQAPK

SEQ ID NO: 36 - protein, 58 aa, synthetic construct
  REGION 1..58: note = cs24 43C
IAAQHDKEQQAAFYEILHLPNLTEDQRNAFIQSLRDDPSVSLCILGEAKKLNDAQAPK

SEQ ID NO: 37 - protein, 58 aa, synthetic construct
  REGION 1..58: note = cs24 46C
IAAQHDKEQQAAFYEILHLPNLTEDQRNAFIQSLRDDPSVSLEILCEAKKLNDAQAPK

SEQ ID NO: 38 - protein, 58 aa, synthetic construct
  REGION 1..58: note = cs24 47C
IAAQHDKEQQAAFYEILHLPNLTEDQRNAFIQSLRDDPSVSLEILGCAKKLNDAQAPK

SEQ ID NO: 39 - protein, 58 aa, synthetic construct
  REGION 1..58: note = cs24 11S 46C
IAAQHDKEQQSAFYEILHLPNLTEDQRNAFIQSLRDDPSVSLEILCEAKKLNDAQAPK

SEQ ID NO: 40 - protein, 58 aa, synthetic construct
  REGION 1..58: note = cs47h3 43C
IAAKHDKDQQAAFYEILHLPNLTEDQRNAFIQSLRDDPSVSLCVLGEAQKLNDSQAPK

SEQ ID NO: 41 - protein, 58 aa, synthetic construct
  REGION 1..58: note = cs47h3 46C
IAAKHDKDQQAAFYEILHLPNLTEDQRNAFIQSLRDDPSVSLEVLCEAQKLNDSQAPK

SEQ ID NO: 42 - protein, 58 aa, synthetic construct
  REGION 1..58: note = cs47h3 47C
IAAKHDKDQQAAFYEILHLPNLTEDQRNAFIQSLRDDPSVSLEVLGCAQKLNDSQAPK

SEQ ID NO: 43 - protein, 58 aa, synthetic construct
  REGION 1..58: note = cs47h3 11S 46C
IAAKHDKDQQSAFYEILHLPNLTEDQRNAFIQSLRDDPSVSLEVLCEAQKLNDSQAPK

SEQ ID NO: 44 - protein, 58 aa, synthetic construct
  REGION 1..58: note = cs47h4 43C
IAAKHDKDQQAAFYEILHLPNLTEEQRNAFIQSLRDDPSVSLCVLGEAQKLNDSQAPK

SEQ ID NO: 45 - protein, 58 aa, synthetic construct
  REGION 1..58: note = cs47h4 46C
IAAKHDKDQQAAFYEILHLPNLTEEQRNAFIQSLRDDPSVSLEVLCEAQKLNDSQAPK

SEQ ID NO: 46 - protein, 58 aa, synthetic construct
  REGION 1..58: note = cs47h4 47C
IAAKHDKDQQAAFYEILHLPNLTEEQRNAFIQSLRDDPSVSLEVLGCAQKLNDSQAPK

SEQ ID NO: 47 - protein, 58 aa, synthetic construct
  REGION 1..58: note = cs74h1 43C
IAAKFDEAQQAAFYEILHLPNLTEDQRNAFIQSLRDDPSVSLCILGEAKKLNDAQAPP

SEQ ID NO: 48 - protein, 58 aa, synthetic construct
  REGION 1..58: note = cs74h1 46C
IAAKFDEAQQAAFYEILHLPNLTEDQRNAFIQSLRDDPSVSLEILCEAKKLNDAQAPP

SEQ ID NO: 49 - protein, 58 aa, synthetic construct
  REGION 1..58: note = cs74h1 47C
IAAKFDEAQQAAFYEILHLPNLTEDQRNAFIQSLRDDPSVSLEILGCAKKLNDAQAPP

SEQ ID NO: 50 - protein, 58 aa, synthetic construct
  REGION 1..58: note = cs74h2 43C
IAAKFDEAQQAAFYEILHLPNLTEEQRNAFIQSLRDDPSVSLCILGEAKKLNDAQAPP

SEQ ID NO: 51 - protein, 58 aa, synthetic construct
  REGION 1..58: note = cs74h2 46C
IAAKFDEAQQAAFYEILHLPNLTEEQRNAFIQSLRDDPSVSLEILCEAKKLNDAQAPP

SEQ ID NO: 52 - protein, 58 aa, synthetic construct
  REGION 1..58: note = cs74h2 47C
IAAKFDEAQQAAFYEILHLPNLTEEQRNAFIQSLRDDPSVSLEILGCAKKLNDAQAPP

SEQ ID NO: 53 - protein, 58 aa, synthetic construct
  REGION 1..58: note = cs20 46C
IDSKFDEAQQAAFYEILHLPSLTEDQRNAFIQSLRDDPSTSLSLLCEAKKLNDAQAPP

SEQ ID NO: 54 - protein, 58 aa, synthetic construct
  REGION 1..58: note = cs20 43C
IDSKFDEAQQAAFYEILHLPSLTEDQRNAFIQSLRDDPSTSLCLLGEAKKLNDAQAPP

SEQ ID NO: 55 - protein, 58 aa, synthetic construct
  REGION 1..58: note = cs20 47C
IDSKFDEAQQAAFYEILHLPSLTEDQRNAFIQSLRDDPSTSLSLLGCAKKLNDAQAPP

SEQ ID NO: 56 - protein, 58 aa, synthetic construct
  REGION 1..58: note = cs20 11S 46C
IDSKFDEAQQSAFYEILHLPSLTEDQRNAFIQSLRDDPSTSLSLLCEAKKLNDAQAPP

SEQ ID NO: 57 - protein, 58 aa, synthetic construct
  REGION 1..58: note = cs17 46C
IDSKFDEAQQAAFYEILHLPNLTEDQRNAFIQSLRDDPSVSLSLLCEAKKLNDAQAPP

SEQ ID NO: 58 - protein, 58 aa, synthetic construct
  REGION 1..58: note = cs42 46C
IDAKHDEDQQAAFYEILHLPNLTEEQRNAFIQSLRDDPSQSLEILCEAKKLNESQAPK

SEQ ID NO: 59 - protein, 58 aa, synthetic construct
  REGION 1..58: note = cs42 47C
IDAKHDEDQQAAFYEILHLPNLTEEQRNAFIQSLRDDPSQSLEILGCAKKLNESQAPK

SEQ ID NO: 60 - protein, 58 aa, synthetic construct
  REGION 1..58: note = cs42 43C
IDAKHDEDQQAAFYEILHLPNLTEEQRNAFIQSLRDDPSQSLCILGEAKKLNESQAPK

SEQ ID NO: 61 - protein, 58 aa, synthetic construct
  REGION 1..58: note = cs42 11S 46C
IDAKHDEDQQSAFYEILHLPNLTEEQRNAFIQSLRDDPSQSLEILCEAKKLNESQAPK

SEQ ID NO: 62 - protein, 58 aa, synthetic construct
  REGION 1..58: note = cs41 46C
IAAKHDEDQQAAFYEILHLPNLTEEQRNAFIQSLRDDPSVSLEILCEAKKLNDSQAPK

SEQ ID NO: 63 - protein, 58 aa, synthetic construct
  REGION 1..58: note = cs28 46C
IDAQHDEDQQAAFYEILHLPNLTEEQRNAFIQSLRDDPSQSLEILCEAKKLNESQAPK

SEQ ID NO: 64 - protein, 58 aa, synthetic construct
  REGION 1..58: note = cs23 46C
IAAKHDKDQQAAFYEILHLPSLTEDQRNAFIQSLRDDPSTSLSILCEAKKLNDAQAPP

SEQ ID NO: 65 - protein, 58 aa, synthetic construct
  REGION 1..58: note = cs25 46C
IAAKHDKDQQAAFYEILHLPNLTEDQRNAFIQSLRDDPSVSLEILCEAKKLNDAQAPK

SEQ ID NO: 66 - protein, 58 aa, synthetic construct
  REGION 1..58: note = cs31 46C
IAAKHDKDQQAAFYEILHLPSLTEDQRNAFIQSLRDDPSVSLEILCEAKKLDDAQAPK

SEQ ID NO: 67 - protein, 58 aa, synthetic construct
  REGION 1..58: note = cs43 46C
IAAKHDKDQQAAFYEILHLPNLTEEQRNAFIQSLRDDPSVSLEILCEAKKLNDSQAPK

SEQ ID NO: 68 - protein, 58 aa, synthetic construct
  REGION 1..58: note = cs44 46C
IAAKHDKDQQAAFYEILHLPNLTEEQRNAFIQSLRDDPSVSLEVLCEAKKLNDAQAPK

SEQ ID NO: 69 - protein, 58 aa, synthetic construct
  REGION 1..58: note = cs45 46C
IAAKHDKDQQAAFYEILHLPSLTEDARNAFIQSLRDDPSVSLEILCEAKKLDDAQAPK

SEQ ID NO: 70 - protein, 58 aa, synthetic construct
  REGION 1..58: note = cs15 46C
IDNKFDEAQQAAFYEILHLPNLTEDQRNAFIQSLRDDPSVSLEILCEAKKLNDAQAPP

SEQ ID NO: 71 - protein, 58 aa, synthetic construct
  REGION 1..58: note = cs16 46C
IDSKFDEAQQAAFYEILHLPNLTEDQRNAFIQSLRDDPSVSLEILCEAKKLNDAQAPP

SEQ ID NO: 72 - protein, 58 aa, synthetic construct
  REGION 1..58: note = cs35 46C
IDAKFDKEQQAAFYEILHLPNLTEEQRNAFIQSLRDDPSQSLELLCEAKKLNDAQAPK

SEQ ID NO: 73 - protein, 61 aa, synthetic construct
  REGION 1..61: note = cs17 11S 46C
IDSIDSKFDEAQQSAFYEILHLPNLTEDQRNAFIQSLRDDPSVSLSLLCEAKKLNDAQAPP

SEQ ID NO: 74 - protein, 58 aa, synthetic construct
  REGION 1..58: note = IB14 43C
PAAKHDKDQQSAFYEILHLPNLTEDQRSAFIQSLKDDPSVSKCILGEAKKLNDAQAPP

SEQ ID NO: 75 - protein, 58 aa, synthetic construct
  REGION 1..58: note = IB14 46C
PAAKHDKDQQSAFYEILHLPNLTEDQRSAFIQSLKDDPSVSKEILCEAKKLNDAQAPP

SEQ ID NO: 76 - protein, 58 aa, synthetic construct
  REGION 1..58: note = IB14 47C
PAAKHDKDQQSAFYEILHLPNLTEDQRSAFIQSLKDDPSVSKEILGCAKKLNDAQAPP

SEQ ID NO: 77 - protein, 58 aa, synthetic construct
  REGION 1..58: note = IB14 50C
PAAKHDKDQQSAFYEILHLPNLTEDQRSAFIQSLKDDPSVSKEILGEAKCLNDAQAPP

SEQ ID NO: 78 - protein, 58 aa, synthetic construct
  REGION 1..58: note = IB14
PAAKHDKDQQSAFYEILHLPNLTEDQRSAFIQSLKDDPSVSKEILGEAKKLNDAQAPP

SEQ ID NO: 79 - protein, 58 aa, synthetic construct
  REGION 1..58: note = IB27
AAAKFDEAQQSAFYEILHLPNLTEEQRNAFIQSLKDDPSVSKEVLGEAQKLNDSQAPK

SEQ ID NO: 80 - protein, 58 aa, synthetic construct
  REGION 1..58: note = IB24
AAAQHDKEQQSAFYEILHLPNLTEDQRNAFIQSLKDDPSVSKEILGEAKKLNDAQAPK

SEQ ID NO: 81 - protein, 58 aa, synthetic construct
  REGION 1..58: note = IB26
AAAQHDKDQQSAFYEILHLPNLTEEQRNAFIQSLKDDPSVSKEILAEAKKLNDAQAPK

SEQ ID NO: 82 - protein, 58 aa, synthetic construct
  REGION 1..58: note = IB28
ADAQHDEDQQSAFYEILHLPNLTEEQRNAFIQSLKDDPSQSKEILGEAKKLNESQAPK

SEQ ID NO: 83 - protein, 58 aa, synthetic construct
  REGION 1..58: note = IB20
ADAKFDEAQQSAFYEILHLPNLTEDQRNAFIQSLKDDPSTSKSLLGEAKKLNDAQAPP

SEQ ID NO: 84 - protein, 58 aa, synthetic construct
  REGION 1..58: note = domain C
ADNKFNKEQQNAFYEILHLPNLTEEQRNGFIQSLKDDPSVSKEILAEAKKLNDAQAPK

SEQ ID NO: 85 - protein, 58 aa, synthetic construct [sequence omitted]

SEQ ID NO: 86 - protein, 58 aa, synthetic construct [sequence omitted]

SEQ ID NO: 87 - protein, 10 aa, synthetic construct
  REGION 1..10: note = spacer
ASPAPSAPSA

SEQ ID NO: 88 - protein, 21 aa, synthetic construct
  REGION 1..21: note = spacer and taq
ASPAPSAPSACASWSHPQFEK

SEQ ID NO: 89 - protein, 8 aa, synthetic construct
  REGION 1..8: note = taq for purification
WSHPQFEK

SEQ ID NO: 90 - protein, 58 aa, synthetic construct
  REGION 1..58: note = cs26 50C
IAAQHDKDQQAAFYEILHLPNLTEEQRNAFIQSLRDDPSVSLEILAEAKCLNDAQAPK

SEQ ID NO: 91 - protein, 58 aa, synthetic construct
  REGION 1..58: note = cs26 51C
IAAQHDKDQQAAFYEILHLPNLTEEQRNAFIQSLRDDPSVSLEILAEAKKCNDAQAPK

SEQ ID NO: 92 - protein, 58 aa, synthetic construct
  REGION 1..58: note = cs26 53C
IAAQHDKDQQAAFYEILHLPNLTEEQRNAFIQSLRDDPSVSLEILAEAKKLNCAQAPK

SEQ ID NO: 93 - protein, 58 aa, synthetic construct
  REGION 1..58: note = cs24 50C
IAAQHDKEQQAAFYEILHLPNLTEDQRNAFIQSLRDDPSVSLEILGEAKCLNDAQAPK

SEQ ID NO: 94 - protein, 58 aa, synthetic construct
  REGION 1..58: note = cs24 51C
IAAQHDKEQQAAFYEILHLPNLTEDQRNAFIQSLRDDPSVSLEILGEAKKCNDAQAPK

SEQ ID NO: 95 - protein, 58 aa, synthetic construct
  REGION 1..58: note = cs24 53C
IAAQHDKEQQAAFYEILHLPNLTEDQRNAFIQSLRDDPSVSLEILGEAKKLNCAQAPK